European Patent Specification EP 3 431 104 B1, published July 22, 2026. Title: STABLE IGG4 BASED BINDING AGENT FORMULATIONS. Applicant: SANOFI. The sequence listing filed with the application follows.

SEQUENCE LISTING (29 sequences)

SEQ ID NO: 1 - protein, 5 aa, Artificial Sequence
  source: /note="Description of Artificial Sequence: Synthetic peptide"
GYNWH

SEQ ID NO: 2 - protein, 16 aa, Artificial Sequence
  source: /note="Description of Artificial Sequence: Synthetic peptide"
EITHSGSTNYNPSLKS

SEQ ID NO: 3 - protein, 14 aa, Artificial Sequence
  source: /note="Description of Artificial Sequence: Synthetic peptide"
EIAVAGTGYYGMDV

SEQ ID NO: 4 - protein, 11 aa, Artificial Sequence
  source: /note="Description of Artificial Sequence: Synthetic peptide"
RASQGINSAFA

SEQ ID NO: 5 - protein, 7 aa, Artificial Sequence
  source: /note="Description of Artificial Sequence: Synthetic peptide"
DASSLES

SEQ ID NO: 6 - protein, 9 aa, Artificial Sequence
  source: /note="Description of Artificial Sequence: Synthetic peptide"
QQFNSYPLT

SEQ ID NO: 7 - protein, 448 aa, Artificial Sequence
  source: /note="Description of Artificial Sequence: Synthetic polypeptide"
QVQLQQWGAGLLKPSETLSLTCAVYGGSFSGYNWHWIRQPPGKGLEWIGEITHSGSTNYNPSLKSRVTISVDTSKNQFSLKLSSVTAADTAVYYCVREIAVAGTGYYGMDVWGQGTTVTVSSASTKGPSVFPLAPCSRSTSESTAALGCLVKDYFPEPVTVSWNSGALTSGVHTFPAVLQSSGLYSLSSVVTVPSSSLGTKTYTCNVDHKPSNTKVDKRVESKYGPPCPPCPAPEFEGGPSVFLFPPKPKDTLMISRTPEVTCVVVDVSQEDPEVQFNWYVDGVEVHNAKTKPREEQFNSTYRVVSVLTVLHQDWLNGKEYKCKVSNKGLPSSIEKTISKAKGQPREPQVYTLPPSQEEMTKNQVSLTCLVKGFYPSDIAVEWESNGQPENNYKTTPPVLDSDGSFFLYSRLTVDKSRWQEGNVFSCSVMHEALHNHYTQKSLSLSLG

SEQ ID NO: 8 - protein, 214 aa, Artificial Sequence
  source: /note="Description of Artificial Sequence: Synthetic polypeptide"
AIQLTQSPSSLSASVGDRVTITCRASQGINSAFAWYQQKPGKAPKLLIYDASSLESGVPSRFSGSGSGTDFTLTISSLQPEDFATYYCQQFNSYPLTFGGGTKVEIKRTVAAPSVFIFPPSDEQLKSGTASVVCLLNNFYPREAKVQWKVDNALQSGNSQESVTEQDSKDSTYSLSSTLTLSKADYEKHKVYACEVTHQGLSSPVTKSFNRGEC

SEQ ID NO: 9 - protein, 240 aa, Homo sapiens
MEESVVRPSVFVVDGQTDIPFTRLGRSHRRQSCSVARVGLGLLLLLMGAGLAVQGWFLLQLHWRLGEMVTRLPDGPAGSWEQLTQERRSHEVNPAAHLTGANSSLTGSGGPLLWETQLGLAFLRGLSYHDGALVVTKAGYYYIYSKVQLGGVGCPLGLASTITHGLYKRTPRYPEELELLVSQQSPCGRATSSSRVWWDSSFLGGVVHLEAGEEVVVRVLDERLVRLRDGTRSYFGAFMV

SEQ ID NO: 10 - protein, 467 aa, Artificial Sequence
  source: /note="Description of Artificial Sequence: Synthetic polypeptide"
MKHLWFFLLLVAAPRWVLSQVQLQQWGAGLLKPSETLSLTCAVYGGSFSGYNWHWIRQPPGKGLEWIGEITHSGSTNYNPSLKSRVTISVDTSKNQFSLKLSSVTAADTAVYYCVREIAVAGTGYYGMDVWGQGTTVTVSSASTKGPSVFPLAPCSRSTSESTAALGCLVKDYFPEPVTVSWNSGALTSGVHTFPAVLQSSGLYSLSSVVTVPSSSLGTKTYTCNVDHKPSNTKVDKRVESKYGPPCPPCPAPEFEGGPSVFLFPPKPKDTLMISRTPEVTCVVVDVSQEDPEVQFNWYVDGVEVHNAKTKPREEQFNSTYRVVSVLTVLHQDWLNGKEYKCKVSNKGLPSSIEKTISKAKGQPREPQVYTLPPSQEEMTKNQVSLTCLVKGFYPSDIAVEWESNGQPENNYKTTPPVLDSDGSFFLYSRLTVDKSRWQEGNVFSCSVMHEALHNHYTQKSLSLSLG

SEQ ID NO: 11 - DNA, 1404 bp, Artificial Sequence
  source: /note="Description of Artificial Sequence: Synthetic polynucleotide"
  CDS (1)..(1401)
atgaagcacctgtggttctttctgctgctggtggccgctcctagatgggtgctgtcccaggtgcagctgcagcagtggggcgctggcctgctgaagccttccgagacactgtccctgacctgcgccgtgtacggcggctccttctccggctacaactggcactggatcaggcagcctcccggcaagggcctggaatggatcggcgagatcacccactccggctccaccaactacaaccctagcctgaagtccagagtgaccatctccgtggacacctccaagaaccagttctccctgaagctgtcctctgtgaccgccgctgacaccgccgtgtactactgtgtgcgggagatcgccgtggctggcaccggctactacggcatggatgtgtggggccagggcaccaccgtgaccgtgtccagcgcttctaccaagggcccttccgtgttccctctggccccttgctcccggtccacctccgagtccaccgccgctctgggctgcctggtgaaggactacttccctgagcctgtgaccgtgtcctggaactctggcgccctgacctccggcgtgcacaccttccctgccgtgctgcagtcctccggcctgtactccctgtcctccgtggtgaccgtgccttcctcctccctgggcaccaagacctacacctgtaacgtggaccacaagccttccaacaccaaggtggacaagcgggtggagtccaagtacggccctccttgccctccctgccctgcccctgagttcgagggcggacctagcgtgttcctgttccctcctaagcctaaggacaccctgatgatctcccggacccctgaggtgacctgtgtggtggtggacgtgtcccaggaggaccctgaggtccagttcaactggtacgtggacggcgtggaggtgcacaacgccaagaccaagcctcgggaggagcagttcaattccacctaccgggtggtgtctgtgctgaccgtgctgcaccaggactggctgaacggcaaagaatacaagtgtaaggtctccaacaagggcctgccctcctccatcgagaaaaccatctccaaggccaagggccagcctagggagcctcaggtgtacaccctgcctcctagccaggaagagatgaccaagaaccaggtgtccctgacctgtctggtgaagggcttctacccttccgacatcgccgtggagtgggagtccaacggccagcctgagaacaactacaagaccacccctcctgtgctggactccgacggctccttcttcctgtactccaggctgaccgtggacaagtcccggtggcaggagggcaacgtcttttcctgctccgtgatgcacgaggccctgcacaaccactacacccagaagtccctgtccctgtctctgggctga

SEQ ID NO: 12 - protein, 236 aa, Artificial Sequence
  source: /note="Description of Artificial Sequence: Synthetic polypeptide"
MDMRVPAQLLGLLLLWLPGARCAIQLTQSPSSLSASVGDRVTITCRASQGINSAFAWYQQKPGKAPKLLIYDASSLESGVPSRFSGSGSGTDFTLTISSLQPEDFATYYCQQFNSYPLTFGGGTKVEIKRTVAAPSVFIFPPSDEQLKSGTASVVCLLNNFYPREAKVQWKVDNALQSGNSQESVTEQDSKDSTYSLSSTLTLSKADYEKHKVYACEVTHQGLSSPVTKSFNRGEC

SEQ ID NO: 13 - DNA, 711 bp, Artificial Sequence
  source: /note="Description of Artificial Sequence: Synthetic polynucleotide"
  CDS (1)..(708)
atggacatgagagtgcctgctcagctgctgggactgctgctgctgtggctgcctggcgctagatgcgccatccagctgacccagtccccctcctctctgtccgcctccgtgggcgacagagtgaccatcacctgtcgggcctcccagggcatcaactccgccttcgcctggtatcagcagaagcctggcaaggcccctaagctgctgatctacgacgcctcctccctggaatccggcgtgccctccagattttccggctccggctctggcaccgacttcaccctgaccatctccagcctgcagcctgaggacttcgccacctactactgccagcagttcaactcctaccctctgaccttcggcggaggcaccaaggtggagatcaagcgtacggtggctgcaccatctgtcttcatcttcccgccatctgatgagcagttgaaatctggaactgcctctgttgtgtgcctgctgaataacttctatcccagagaggccaaagtacagtggaaggtggataacgccctccaatcgggtaactcccaggagagtgtcacagagcaggacagcaaggacagcacctacagcctcagcagcaccctgacgctgagcaaagcagactacgagaaacacaaagtctacgcctgcgaagtcacccatcagggcctgagctcgcccgtcacaaagagcttcaacaggggagagtgttag

SEQ ID NO: 14 - protein, 372 aa, Homo sapiens
MNYPLTLEMDLENLEDLFWELDRLDNYNDTSLVENHLCPATEGPLMASFKAVFVPVAYSLIFLLGVIGNVLVLVILERHRQTRSSTETFLFHLAVADLLLVFILPFAVAEGSVGWVLGTFLCKTVIALHKVNFYCSSLLLACIAVDRYLAIVHAVHAYRHRRLLSIHITCGTIWLVGFLLALPEILFAKVSQGHHNNSLPRCTFSQENQAETHAWFTSRFLYHVAGFLLPMLVMGWCYVGVVHRLRQAQRRPQRQKAVRVAILVTSIFFLCWSPYHIVIFLDTLARLKAVDNTCKLNGSLPVAITMCEFLGLAHCCLNPMLYTFAGVKFRSDLSRLLTKLGCTGPASLCQLFPSWRRSSLSESENATSLTTF

SEQ ID NO: 15 - protein, 10 aa, Artificial Sequence
  source: /note="Description of Artificial Sequence: Synthetic peptide"
GFSLIDYGVN

SEQ ID NO: 16 - protein, 9 aa, Artificial Sequence
  source: /note="Description of Artificial Sequence: Synthetic peptide"
VIWGDGTTY

SEQ ID NO: 17 - protein, 3 aa, Artificial Sequence
  source: /note="Description of Artificial Sequence: Synthetic peptide"
IVY

SEQ ID NO: 18 - protein, 16 aa, Artificial Sequence
  source: /note="Description of Artificial Sequence: Synthetic peptide"
RSSKSLLHSSGKTYLY

SEQ ID NO: 19 - protein, 6 aa, Artificial Sequence
  source: /note="Description of Artificial Sequence: Synthetic peptide"
RLSSLA

SEQ ID NO: 20 - protein, 9 aa, Artificial Sequence
  source: /note="Description of Artificial Sequence: Synthetic peptide"
MQHLEYPYT

SEQ ID NO: 21 - protein, 111 aa, Artificial Sequence
  source: /note="Description of Artificial Sequence: Synthetic polypeptide"
QVQLKESGPGLVAPSESLSITCTVSGFSLIDYGVNWIRQPPGKGLEWLGVIWGDGTTYYNPSLKSRLSISKDNSKSQVFLKVTSLTTDDTAMYYCARIVYWGQGTLVTVSA

SEQ ID NO: 22 - protein, 112 aa, Artificial Sequence
  source: /note="Description of Artificial Sequence: Synthetic polypeptide"
DIVMTQAAPSVAVTPGASVSISCRSSKSLLHSSGKTYLYWFLQRPGQSPQLLIYRLSSLASGVPDRFSGSGSGTAFTLRISRVEAEDVGVYYCMQHLEYPYTFGGGTKLEIK

SEQ ID NO: 23 - protein, 326 aa, Artificial Sequence
  source: /note="Description of Artificial Sequence: Synthetic polypeptide"
ASTKGPSVFPLAPCSRSTSESTAALGCLVKDYFPEPVTVSWNSGALTSGVHTFPAVLQSSGLYSLSSVVTVPSSSLGTKTYTCNVDHKPSNTKVDKRVESKYGPPCPPCPAPEFEGGPSVFLFPPKPKDTLMISRTPEVTCVVVDVSQEDPEVQFNWYVDGVEVHNAKTKPREEQFNSTYRVVSVLTVLHQDWLNGKEYKCKVSNKGLPSSIEKTISKAKGQPREPQVYTLPPSQEEMTKNQVSLTCLVKGFYPSDIAVEWESNGQPENNYKTTPPVLDSDGSFFLYSRLTVDKSRWQEGNVFSCSVMHEALHNHYTQKSLSLSLG

SEQ ID NO: 24 - protein, 107 aa, Artificial Sequence [sequence omitted]

SEQ ID NO: 25 - protein, 437 aa, Artificial Sequence
  source: /note="Description of Artificial Sequence: Synthetic polypeptide"
QVQLKESGPGLVAPSESLSITCTVSGFSLIDYGVNWIRQPPGKGLEWLGVIWGDGTTYYNPSLKSRLSISKDNSKSQVFLKVTSLTTDDTAMYYCARIVYWGQGTLVTVSAASTKGPSVFPLAPCSRSTSESTAALGCLVKDYFPEPVTVSWNSGALTSGVHTFPAVLQSSGLYSLSSVVTVPSSSLGTKTYTCNVDHKPSNTKVDKRVESKYGPPCPPCPAPEFEGGPSVFLFPPKPKDTLMISRTPEVTCVVVDVSQEDPEVQFNWYVDGVEVHNAKTKPREEQFNSTYRVVSVLTVLHQDWLNGKEYKCKVSNKGLPSSIEKTISKAKGQPREPQVYTLPPSQEEMTKNQVSLTCLVKGFYPSDIAVEWESNGQPENNYKTTPPVLDSDGSFFLYSRLTVDKSRWQEGNVFSCSVMHEALHNHYTQKSLSLSLG

SEQ ID NO: 26 - protein, 219 aa, Artificial Sequence
  source: /note="Description of Artificial Sequence: Synthetic polypeptide"
DIVMTQAAPSVAVTPGASVSISCRSSKSLLHSSGKTYLYWFLQRPGQSPQLLIYRLSSLASGVPDRFSGSGSGTAFTLRISRVEAEDVGVYYCMQHLEYPYTFGGGTKLEIKRTVAAPSVFIFPPSDEQLKSGTASVVCLLNNFYPREAKVQWKVDNALQSGNSQESVTEQDSKDSTYSLSSTLTLSKADYEKHKVYACEVTHQGLSSPVTKSFNRGEC

SEQ ID NO: 27 - protein, 19 aa, Artificial Sequence
  source: /note="Description of Artificial Sequence: Synthetic peptide"
MGWSCIILFLVATATGVHS

SEQ ID NO: 28 - protein, 456 aa, Artificial Sequence
  source: /note="Description of Artificial Sequence: Synthetic polypeptide"
MGWSCIILFLVATATGVHSQVQLKESGPGLVAPSESLSITCTVSGFSLIDYGVNWIRQPPGKGLEWLGVIWGDGTTYYNPSLKSRLSISKDNSKSQVFLKVTSLTTDDTAMYYCARIVYWGQGTLVTVSAASTKGPSVFPLAPCSRSTSESTAALGCLVKDYFPEPVTVSWNSGALTSGVHTFPAVLQSSGLYSLSSVVTVPSSSLGTKTYTCNVDHKPSNTKVDKRVESKYGPPCPPCPAPEFEGGPSVFLFPPKPKDTLMISRTPEVTCVVVDVSQEDPEVQFNWYVDGVEVHNAKTKPREEQFNSTYRVVSVLTVLHQDWLNGKEYKCKVSNKGLPSSIEKTISKAKGQPREPQVYTLPPSQEEMTKNQVSLTCLVKGFYPSDIAVEWESNGQPENNYKTTPPVLDSDGSFFLYSRLTVDKSRWQEGNVFSCSVMHEALHNHYTQKSLSLSLG

SEQ ID NO: 29 - protein, 238 aa, Artificial Sequence
  source: /note="Description of Artificial Sequence: Synthetic polypeptide"
MGWSCIILFLVATATGVHSDIVMTQAAPSVAVTPGASVSISCRSSKSLLHSSGKTYLYWFLQRPGQSPQLLIYRLSSLASGVPDRFSGSGSGTAFTLRISRVEAEDVGVYYCMQHLEYPYTFGGGTKLEIKRTVAAPSVFIFPPSDEQLKSGTASVVCLLNNFYPREAKVQWKVDNALQSGNSQESVTEQDSKDSTYSLSSTLTLSKADYEKHKVYACEVTHQGLSSPVTKSFNRGEC